European Patent Specification EP 4 138 870 B1, published August 28, 2024. Title: COMPOSITION FOR USE IN THE TREATMENT OF GROUP-B STREPTOCOCCUS (GBS)INFECTIONS. Applicant: GIELLEPI S.P.A. The sequence listing filed with the application follows.

SEQUENCE LISTING (1 sequence)

SEQ ID NO: 1 - DNA, 550 bp, Artificial Sequence
  region from the 16s rRNA gene
tggagagtttgatcctggctcaggacgaacgctggcggcgtgcctaatacatgcaagtcgagcgagctgaaccaacagattcacttcggtgatgacgttgggaacgcgagcggcggatgggtgagtaacacgtggggaacctgccccatagtctgggataccacttggaaacaggtgctaataccggataagaaagcagatcgcatgatcagcttataaaaggcggcgtaagctgtcgctatgggatggccccgcggtgcattagctagttggtagggtaacggcctaccaaggcaatgatgcatagccgagttgagagactgatcggccacattgggactgagacacggcccaaactcctacgggaggcagcagtagggaatcttccacaatggacgaaagtctgatggagcaacgccgcgtgagtgaagaaggttttcggatcgtaaagctctgttgttggtgaagaaggatagaggtagtaactggcctttatttgacggtaatcaaccagaaagtcacggctaactacgtgccagcagccgcggta